European Patent Application EP 4 403 629 A1, published July 24, 2024. Title: Novel Acetohydroxy acid synthase variant and method of producing L-isoleucine using the same. Applicant: CJ CheilJedang Corporation. The sequence listing filed with the application follows.

SEQUENCE LISTING (24 sequences)

SEQ ID NO: 1 - protein, 172 aa, Corynebacterium sp.
  REGION 1..172: note = ilvN
MANSDVTRHILSVLVQDVDGIISRVSGMFTRRAFNLVSLVSAKTETHGINRITVVVDADELNIEQITKQLNKLIPVLKVVRLDEETTIARAIMLVKVSADSTNRPQIVDAANIFRARVVDVAPDSVVIESTGTPGKLRALLDVMEPFGIRELIQSGQIALNRGPKTMAPAKI

SEQ ID NO: 2 - DNA, 519 bp, Corynebacterium sp.
  misc_feature 1..519: note = ilvN
  source 1..519: mol_type = genomic DNA
atggctaattctgacgtcacccgccacatcctgtccgtactcgttcaggacgtagacggaatcatttcccgcgtatcaggtatgttcacccgacgcgcattcaacctcgtgtccctcgtgtctgcaaagaccgaaacacacggcatcaaccgcatcacggttgttgtcgacgccgacgagctcaacattgagcagatcaccaagcagctcaacaagctgatccccgtgctcaaagtcgtgcgacttgatgaagagaccactatcgcccgcgcaatcatgctggttaaggtctctgcggacagcaccaaccgtccgcagatcgtcgacgccgcgaacatcttccgcgcccgagtcgtcgacgtggctccagactctgtggttattgaatccacaggcaccccaggcaagctccgcgcactgcttgacgtgatggaaccattcggaatccgcgaactgatccaatccggacagattgcactcaaccgcggtccgaagaccatggctccggccaagatctaa

SEQ ID NO: 3 - protein, 172 aa, synthetic construct
  REGION 1..172: note = ilvN(A42V)
MANSDVTRHILSVLVQDVDGIISRVSGMFTRRAFNLVSLVSVKTETHGINRITVVVDADELNIEQITKQLNKLIPVLKVVRLDEETTIARAIMLVKVSADSTNRPQIVDAANIFRARVVDVAPDSVVIESTGTPGKLRALLDVMEPFGIRELIQSGQIALNRGPKTMAPAKI

SEQ ID NO: 4 - protein, 172 aa, synthetic construct
  REGION 1..172: note = ilvN(H47L)
MANSDVTRHILSVLVQDVDGIISRVSGMFTRRAFNLVSLVSAKTETLGINRITVVVDADELNIEQITKQLNKLIPVLKVVRLDEETTIARAIMLVKVSADSTNRPQIVDAANIFRARVVDVAPDSVVIESTGTPGKLRALLDVMEPFGIRELIQSGQIALNRGPKTMAPAKI

SEQ ID NO: 5 - protein, 172 aa, synthetic construct
  REGION 1..172: note = ilvN(A42V, H47L)
MANSDVTRHILSVLVQDVDGIISRVSGMFTRRAFNLVSLVSVKTETLGINRITVVVDADELNIEQITKQLNKLIPVLKVVRLDEETTIARAIMLVKVSADSTNRPQIVDAANIFRARVVDVAPDSVVIESTGTPGKLRALLDVMEPFGIRELIQSGQIALNRGPKTMAPAKI

SEQ ID NO: 6 - DNA, 35 bp, synthetic construct
  misc_feature 1..35: note = primer 1
  source 1..35: mol_type = other DNA
tcgagctcggtaccccgcttttgcactcatcgagc

SEQ ID NO: 7 - DNA, 23 bp, synthetic construct
  misc_feature 1..23: note = primer 2
  source 1..23: mol_type = other DNA
cacgatcagatgtgcatcatcat

SEQ ID NO: 8 - DNA, 23 bp, synthetic construct
  misc_feature 1..23: note = primer 3
  source 1..23: mol_type = other DNA
atgatgatgcacatctgatcgtg

SEQ ID NO: 9 - DNA, 35 bp, synthetic construct
  misc_feature 1..35: note = primer 4
  source 1..35: mol_type = other DNA
ctctagaggatccccgagcatcttccaaaaccttg

SEQ ID NO: 10 - DNA, 35 bp, synthetic construct
  misc_feature 1..35: note = primer 5
  source 1..35: mol_type = other DNA
tcgagctcggtacccatgagtgaaacatacgtgtc

SEQ ID NO: 11 - DNA, 39 bp, synthetic construct
  misc_feature 1..39: note = primer 6
  source 1..39: mol_type = other DNA
gcgcttgaggtactctgccagcgcgatgtcatcatccgg

SEQ ID NO: 12 - DNA, 39 bp, synthetic construct
  misc_feature 1..39: note = primer 7
  source 1..39: mol_type = other DNA
ccggatgatgacatcgcgctggcagagtacctcaagcgc

SEQ ID NO: 13 - DNA, 34 bp, synthetic construct
  misc_feature 1..34: note = primer 8
  source 1..34: mol_type = other DNA
ctctagaggatcccccgtcaccgacacctccaca

SEQ ID NO: 14 - DNA, 30 bp, synthetic construct
  misc_feature 1..30: note = primer 9
  source 1..30: mol_type = other DNA
cgagctcggtacccatggctaattctgacg

SEQ ID NO: 15 - DNA, 30 bp, synthetic construct
  misc_feature 1..30: note = primer 10
  source 1..30: mol_type = other DNA
tagaggatccccttagatcttggccggagc

SEQ ID NO: 16 - DNA, 1338 bp, synthetic construct
  misc_feature 1..1338: note = hom(R407H)
  source 1..1338: mol_type = other DNA
atgacctcagcatctgccccaagctttaaccccggcaagggtcccggctcagcagtcggaattgcccttttaggattcggaacagtcggcactgaggtgatgcgtctgatgaccgagtacggtgatgaacttgcgcaccgcattggtggcccactggaggttcgtggcattgctgtttctgatatctcaaagccacgtgaaggcgttgcacctgagctgctcactgaggacgcttttgcactcatcgagcgcgaggatgttgacatcgtcgttgaggttatcggcggcattgagtacccacgtgaggtagttctcgcagctctgaaggccggcaagtctgttgttaccgccaataaggctcttgttgcagctcactctgctgagcttgctgatgcagcggaagccgcaaacgttgacctgtacttcgaggctgctgttgcaggcgcaattccagtggttggcccactgcgtcgctccctggctggcgatcagatccagtctgtgatgggcatcgttaacggcaccaccaacttcatcttggacgccatggattccaccggcgctgactatgcagattctttggctgaggcaactcgtttgggttacgccgaagctgatccaactgcagacgtcgaaggccatgacgccgcatccaaggctgcaattttggcatccatcgctttccacacccgtgttaccgcggatgatgtgtactgcgaaggtatcagcaacatcagcgctgccgacattgaggcagcacagcaggcaggccacaccatcaagttgttggccatctgtgagaagttcaccaacaaggaaggaaagtcggctatttctgctcgcgtgcacccgactctattacctgtgtcccacccactggcgtcggtaaacaagtcctttaatgcaatctttgttgaagcagaagcagctggtcgcctgatgttctacggaaacggtgcaggtggcgcgccaaccgcgtctgctgtgcttggcgacgtcgttggtgccgcacgaaacaaggtgcacggtggccgtgctccaggtgagtccacctacgctaacctgccgatcgctgatttcggtgagaccaccactcgttaccacctcgacatggatgtggaagatcgcgtgggggttttggctgaattggctagcctgttctctgagcaaggaatctccctgcgtacaatccgacaggaagagcgcgatgatgatgcacatctgatcgtggtcacccactctgcgctggaatctgatctttcccgcaccgttgaactgctgaaggctaagcctgttgttaaggcaatcaacagtgtgatccgcctcgaaagggactaa

SEQ ID NO: 17 - DNA, 1311 bp, synthetic construct
  misc_feature 1..1311: note = ilvA(T381A, F383A)
  source 1..1311: mol_type = other DNA
atgagtgaaacatacgtgtctgagaaaagtccaggagtgatggctagcggagcggagctgattcgtgccgccgacattcaaacggcgcaggcacgaatttcctccgtcattgcaccaactccattgcagtattgccctcgtctttctgaggaaaccggagcggaaatctaccttaagcgtgaggatctgcaggatgttcgttcctacaagatccgcggtgcgctgaactctggagcgcagctcactcaggagcagcgcgatgcaggtatcgttgccgcatctgcaggtaaccatgcccagggcgtggcctatgtgtgcaagtccttgggcgttcagggacgcatctatgttcctgtgcagactccaaagcaaaagcgtgaccgcatcatggttcacggcggagagtttgtctccttggtggtcactggcaataacttcgacgaagcatcggctgcagcgcatgaagatgcagagcgcaccggcgcaacgctgatcgagcctttcgatgctcgcaacaccgtcatcggtcagggtacagtggctgctgagatcttgtcgcagctgacttccatgggcaagagtgcagatcacgtgatggttccagtcggcggtggcggacttcttgcaggtgtggtcagctacatggctgatatggcacctcgcactgcgatcgttggtatcgaaccagcgggagcagcatccatgcaggctgcattgcacaatggtggaccaatcactttggagactgttgatccctttgtggacggcgcagcagtcaaacgtgtcggagatctcaactacaccatcgtggagaagaaccagggtcgcgtgcacatgatgagcgcgaccgagggcgctgtgtgtactgagatgctcgatctttaccaaaacgaaggcatcatcgcggagcctgctggcgcgctgtctatcgctgggttgaaggaaatgtcctttgcacctggttctgtcgtggtgtgcatcatctctggtggcaacaacgatgtgctgcgttatgcggaaatcgctgagcgctccttggtgcaccgcggtttgaagcactacttcttggtgaacttcccgcaaaagcctggtcagttgcgtcacttcctggaagatatcctgggaccggatgatgacatcgcgctggcagagtacctcaagcgcaacaaccgtgagaccggtactgcgttggtgggtattcacttgagtgaagcatcaggattggattctttgctggaacgtatggaggaatcggcaattgattcccgtcgcctcgagccgggcacccctgagtacgaatacttgacctaa

SEQ ID NO: 18 - DNA, 30 bp, synthetic construct
  misc_feature 1..30: note = primer 11
  source 1..30: mol_type = other DNA
ttcggtcttaacagacacgagggacacgag

SEQ ID NO: 19 - DNA, 30 bp, synthetic construct
  misc_feature 1..30: note = primer 12
  source 1..30: mol_type = other DNA
gtgtccctcgtgtctgttaagaccgaaaca

SEQ ID NO: 20 - DNA, 30 bp, synthetic construct
  misc_feature 1..30: note = primer 13
  source 1..30: mol_type = other DNA
cggttgatgccgagtgtttcggtctttgca

SEQ ID NO: 21 - DNA, 30 bp, synthetic construct
  misc_feature 1..30: note = primer 14
  source 1..30: mol_type = other DNA
aagaccgaaacactcggcatcaaccgcatc

SEQ ID NO: 22 - DNA, 519 bp, synthetic construct
  misc_feature 1..519: note = ilvN(A42V)
  source 1..519: mol_type = other DNA
atggctaattctgacgtcacccgccacatcctgtccgtactcgttcaggacgtagacggaatcatttcccgcgtatcaggtatgttcacccgacgcgcattcaacctcgtgtccctcgtgtctgttaagaccgaaacacacggcatcaaccgcatcacggttgttgtcgacgccgacgagctcaacattgagcagatcaccaagcagctcaacaagctgatccccgtgctcaaagtcgtgcgacttgatgaagagaccactatcgcccgcgcaatcatgctggttaaggtctctgcggacagcaccaaccgtccgcagatcgtcgacgccgcgaacatcttccgcgcccgagtcgtcgacgtggctccagactctgtggttattgaatccacaggcaccccaggcaagctccgcgcactgcttgacgtgatggaaccattcggaatccgcgaactgatccaatccggacagattgcactcaaccgcggtccgaagaccatggctccggccaagatctaa

SEQ ID NO: 23 - DNA, 519 bp, synthetic construct
  misc_feature 1..519: note = ilvN(H47L)
  source 1..519: mol_type = other DNA
atggctaattctgacgtcacccgccacatcctgtccgtactcgttcaggacgtagacggaatcatttcccgcgtatcaggtatgttcacccgacgcgcattcaacctcgtgtccctcgtgtctgcaaagaccgaaacactcggcatcaaccgcatcacggttgttgtcgacgccgacgagctcaacattgagcagatcaccaagcagctcaacaagctgatccccgtgctcaaagtcgtgcgacttgatgaagagaccactatcgcccgcgcaatcatgctggttaaggtctctgcggacagcaccaaccgtccgcagatcgtcgacgccgcgaacatcttccgcgcccgagtcgtcgacgtggctccagactctgtggttattgaatccacaggcaccccaggcaagctccgcgcactgcttgacgtgatggaaccattcggaatccgcgaactgatccaatccggacagattgcactcaaccgcggtccgaagaccatggctccggccaagatctaa

SEQ ID NO: 24 - DNA, 519 bp, synthetic construct
  misc_feature 1..519: note = ilvN(A42V, H47L)
  source 1..519: mol_type = other DNA
atggctaattctgacgtcacccgccacatcctgtccgtactcgttcaggacgtagacggaatcatttcccgcgtatcaggtatgttcacccgacgcgcattcaacctcgtgtccctcgtgtctgttaagaccgaaacactcggcatcaaccgcatcacggttgttgtcgacgccgacgagctcaacattgagcagatcaccaagcagctcaacaagctgatccccgtgctcaaagtcgtgcgacttgatgaagagaccactatcgcccgcgcaatcatgctggttaaggtctctgcggacagcaccaaccgtccgcagatcgtcgacgccgcgaacatcttccgcgcccgagtcgtcgacgtggctccagactctgtggttattgaatccacaggcaccccaggcaagctccgcgcactgcttgacgtgatggaaccattcggaatccgcgaactgatccaatccggacagattgcactcaaccgcggtccgaagaccatggctccggccaagatctaa